European Patent Specification EP 3 385 385 B1, published January 11, 2023. Title: Use of Tobacco Gene NtTCTP in Plant against Potato Virus Y. Applicant: Guizhou Institute of Tobacco Science. The sequence listing filed with the application follows.

SEQUENCE LISTING (3 sequences)

SEQ ID NO: 1 - DNA, 507 bp, tobacco
atgttggtttatcaggatcttctctccggtgatgagctcctttcggattcattttcctacactgaacttgagaatggagtgctttgggaagtgcaagggaagtgggttgttcagggagctgttgatgtgaacatcggggcgaatccatctgctgaaggtgcagatgaagacgaaggtgttgacgatcaagccatcaaggttgtcgatattgttgacactttcaggcttcaggagcaaccttcttttgacaagaagcagtttgttgcctacatgaagaaatatatcaagaacctaacacccaagttaggcgcagagcaggaagaagtttttaagaacaacattcaaggagcaaccaagtaccttttgtcaaagctcagtgaccttcaattctttgttggtgagagcatggctgatgatactggaatggtgtttgcctactacaaggatggcgccactgatcctacctttttgtacctcgcacatggactcaaggaggtcaagtgttaa

SEQ ID NO: 2 - protein, 168 aa, tobacco
MLVYQDLLSGDELLSDSFSYTELENGVLWEVQGKWVVQGAVDVNIGANPSAEGADEDEGVDDQAIKVVDIVDTFRLQEQPSFDKKQFVAYMKKYIKNLTPKLGAEQEEVFKNNIQGATKYLLSKLSDLQFFVGESMADDTGMVFAYYKDGATDPTFLYLAHGLKEVKC

SEQ ID NO: 3 - DNA, 782 bp, Artificial sequence
ggatccatgttggtttatcaggatcttctctccggtgatgagctcctttcggattcattttcctacactgaacttgagaatggagtgctttgggaagtgcaagggaagtgggttgttcagggagctgttgatgtgaacatcggggcgaatccatctgctgaaggtgcagatgaagacgaaggtgttgacgatcaagccatcaaggttgtcgatattgttgacactttcaggcttcaggagcaaccttcttttgacaagaagcagtttgttgcctacatgaagaaatatatcaagaacctaacacccaagttaggcgcagagcaggaagaagttttttcaacacctacaccatttttttaatcactactacccattgcattgaacaaacttccaagttcttcttagcttcagattaagaaagtaccctttcttggctttgttgatgtaaaaacttcttcctgctctgcgcctaacttgggtgttaggttcttgatatatttcttcatgtaggcaacaaactgcttcttgtcaaaagaaggttgctcctgaagcctgaaagtgtcaacaatatcgacaaccttgatggcttgatcgtcaacaccttcgtcttcatctgcaccttcagcagatggattcgccccgatgttcacatcaacagctccctgaacaacccacttcccttgcacttcccaaagcactccattctcaagttcagtgtaggaaaatgaatccgaaaggagctcatcaccggagagaagatcctgataaaccaacatgtcgac